European Patent Application EP 4 282 481 A2, published November 29, 2023. Title: SEQUENCES SIARN CIBLANT L'EXPRESSION DES GENES JAK1 OU JAK3 HUMAINS POUR UNE UTILISATION THERAPEUTIQUE. Applicant: Commissariat à l'énergie atomique et aux énergies alternatives. The sequence listing filed with the application follows.

SEQUENCE LISTING (8 sequences)

SEQ ID NO: 1 - RNA, 21 nt, synthetic construct
  misc_feature 1..21: note = brin sens siARN HJD41
  source 1..21: mol_type = other RNA
cgactttccagaaatcgtaga

SEQ ID NO: 2 - RNA, 21 nt, synthetic construct
  misc_feature 1..21: note = brin antisens siARN HJD41
  source 1..21: mol_type = other RNA
tacgatttctggaaagtcgca

SEQ ID NO: 3 - RNA, 21 nt, synthetic construct
  misc_feature 1..21: note = brin sens siARN HMJ3D1
  source 1..21: mol_type = other RNA
gcgtggagctgtgccgctatg

SEQ ID NO: 4 - RNA, 21 nt, synthetic construct
  misc_feature 1..21: note = brin antisens siARN HMJ3D1
  source 1..21: mol_type = other RNA
tagcggcacagctccacgctg

SEQ ID NO: 5 - RNA, 21 nt, synthetic construct
  misc_feature 1..21: note = brin sens siARN HJ1D2
  source 1..21: mol_type = other RNA
ggattacaaggatgacgaagg

SEQ ID NO: 6 - RNA, 21 nt, synthetic construct
  misc_feature 1..21: note = brin antisens siARN HJ1D2
  source 1..21: mol_type = other RNA
ttcgtcatccttgtaatccat

SEQ ID NO: 7 - RNA, 21 nt, synthetic construct
  misc_feature 1..21: note = brin sens siARN HJ1D8
  source 1..21: mol_type = other RNA
ggacatcagctacaagcgata

SEQ ID NO: 8 - RNA, 21 nt, synthetic construct
  misc_feature 1..21: note = brin antisens siARN HJ1D8
  source 1..21: mol_type = other RNA
tcgcttgtagctgatgtcctt